European Patent Application EP 4 729 167 A1, published April 22, 2026. Title: Flow reactor and biological polymer synthesis system comprising the same. Applicant: SP2 TX Inc. The sequence listing filed with the application follows.

SEQUENCE LISTING (1 sequence)

SEQ ID NO: 1 - protein, 10 aa, synthetic construct
VQAAIDYING